European Patent Application EP 4 520 766 A1, published March 12, 2025. Title: 一种靶向卵巢的多肽及其衍生物和应用. Applicant: 中国科学院深圳先进技术研究院. Application WO. The sequence listing filed with the application follows.

SEQUENCE LISTING (10 sequences)

SEQ ID NO: 1 - protein, 15 aa, synthetic construct
YLGASVPSPDPLEPT

SEQ ID NO: 2 - protein, 19 aa, synthetic construct
YLNNGLGAPAPYPDPLEPT

SEQ ID NO: 3 - protein, 19 aa, synthetic construct
YLYQWLGAPVPYPDPLEPT

SEQ ID NO: 4 - protein, 19 aa, synthetic construct
YLYQWLGAPVPYPDTLEPT

SEQ ID NO: 5 - protein, 19 aa, synthetic construct
YLYQWLGAPAPYPDPLEPT

SEQ ID NO: 6 - protein, 19 aa, synthetic construct
YLDHWLGAPAPYPDPLEPT

SEQ ID NO: 7 - protein, 19 aa, synthetic construct
YLDPGLGAPAPYPDPLEPT

SEQ ID NO: 8 - protein, 19 aa, synthetic construct
YLDHGLGAPAPYPDPLEPT

SEQ ID NO: 9 - protein, 19 aa, synthetic construct
YLDQGLGAPAPAPDPLEPT

SEQ ID NO: 10 - protein, 19 aa, synthetic construct
YLDSGLGAPVPYPDPLEPT